European Patent Application EP 4 682 159 A1, published January 21, 2026. Title: Cyclic peptide or salt thereof and use thereof. Applicant: FUJIFILM Corporation. Application WO. The sequence listing filed with the application follows.

SEQUENCE LISTING (346 sequences)

SEQ ID NO: 1 - DNA, 196 bp, synthetic construct
  misc_feature 1..196: note = Description of Artificial Sequence: Artificial DNA
  source 1..196: mol_type = other DNA
gaaattaatacgactcactatagggagaccacaacggtttccctctagaaataattttgtttaactttaagaaggagatatacatatggttaagaaaacaaaaacannntgtnnnnnnnnnnnnnnnnnntagnnnggtggctctggcggtagcaggacggggggcggcggggggtaaataaataagcttgagtat

SEQ ID NO: 2 - DNA, 105 bp, synthetic construct
  misc_feature 1..105: note = Description of Artificial Sequence: Artificial DNA
  source 1..105: mol_type = other DNA
gaaattaatacgactcactatagggagaccacaacggtttccctctagaaataattttgtttaactttaagaaggagatatacatatggttaaaaaaacaaaaac

SEQ ID NO: 3 - DNA, 63 bp, synthetic construct
  misc_feature 1..63: note = Description of Artificial Sequence: Artificial DNA
  source 1..63: mol_type = other DNA
atactcaagcttatttatttattaccccccgccgccccccgtcctgctaccgccagaaccacc

SEQ ID NO: 4 - DNA, 86 bp, synthetic construct
  misc_feature 1..86: note = Description of Artificial Sequence: Artificial DNA
  source 1..86: mol_type = other DNA
aagaaggagatatacatatggttaaaaaaacaaaaacannntgtnnnnnnnnnnnnnnnnnntagnnnggcggttctggcggtagc

SEQ ID NO: 5 - DNA, 89 bp, synthetic construct
  misc_feature 1..89: note = Description of Artificial Sequence: Artificial DNA
  source 1..89: mol_type = other DNA
aagaaggagatatacatatggttaaaaaaacaaaaacannntgtnnnnnnnnnnnnnnnnnnnnntagnnnggcggttctggcggtagc

SEQ ID NO: 6 - DNA, 92 bp, synthetic construct
  misc_feature 1..92: note = Description of Artificial Sequence: Artificial DNA
  source 1..92: mol_type = other DNA
aagaaggagatatacatatggttaaaaaaacaaaaacannntgtnnnnnnnnnnnnnnnnnnnnnnnntagnnnggcggttctggcggtagc

SEQ ID NO: 7 - DNA, 95 bp, synthetic construct
  misc_feature 1..95: note = Description of Artificial Sequence: Artificial DNA
  source 1..95: mol_type = other DNA
aagaaggagatatacatatggttaaaaaaacaaaaacannntgtnnnnnnnnnnnnnnnnnnnnnnnnnnntagnnnggcggttctggcggtagc

SEQ ID NO: 8 - DNA, 98 bp, synthetic construct
  misc_feature 1..98: note = Description of Artificial Sequence: Artificial DNA
  source 1..98: mol_type = other DNA
aagaaggagatatacatatggttaaaaaaacaaaaacannntgtnnnnnnnnnnnnnnnnnnnnnnnnnnnnnntagnnnggcggttctggcggtagc

SEQ ID NO: 9 - DNA, 101 bp, synthetic construct
  misc_feature 1..101: note = Description of Artificial Sequence: Artificial DNA
  source 1..101: mol_type = other DNA
aagaaggagatatacatatggttaaaaaaacaaaaacannntgtnnnnnnnnnnnnnnnnnnnnnnnnnnnnnnnnntagnnnggcggttctggcggtagc

SEQ ID NO: 10 - DNA, 104 bp, synthetic construct
  misc_feature 1..104: note = Description of Artificial Sequence: Artificial DNA
  source 1..104: mol_type = other DNA
aagaaggagatatacatatggttaaaaaaacaaaaacannntgtnnnnnnnnnnnnnnnnnnnnnnnnnnnnnnnnnnnntagnnnggcggttctggcggtagc

SEQ ID NO: 11 - DNA, 107 bp, synthetic construct
  misc_feature 1..107: note = Description of Artificial Sequence: Artificial DNA
  source 1..107: mol_type = other DNA
aagaaggagatatacatatggttaaaaaaacaaaaacannntgtnnnnnnnnnnnnnnnnnnnnnnnnnnnnnnnnnnnnnnntagnnnggcggttctggcggtagc

SEQ ID NO: 12 - DNA, 110 bp, synthetic construct
  misc_feature 1..110: note = Description of Artificial Sequence: Artificial DNA
  source 1..110: mol_type = other DNA
aagaaggagatatacatatggttaaaaaaacaaaaacannntgtnnnnnnnnnnnnnnnnnnnnnnnnnnnnnnnnnnnnnnnnnntagnnnggcggttctggcggtagc

SEQ ID NO: 13 - DNA, 113 bp, synthetic construct
  misc_feature 1..113: note = Description of Artificial Sequence: Artificial DNA
  source 1..113: mol_type = other DNA
aagaaggagatatacatatggttaaaaaaacaaaaacannntgtnnnnnnnnnnnnnnnnnnnnnnnnnnnnnnnnnnnnnnnnnnnnntagnnnggcggttctggcggtagc

SEQ ID NO: 14 - DNA, 116 bp, synthetic construct
  misc_feature 1..116: note = Description of Artificial Sequence: Artificial DNA
  source 1..116: mol_type = other DNA
aagaaggagatatacatatggttaaaaaaacaaaaacannntgtnnnnnnnnnnnnnnnnnnnnnnnnnnnnnnnnnnnnnnnnnnnnnnnntagnnnggcggttctggcggtagc

SEQ ID NO: 15 - DNA, 119 bp, synthetic construct
  misc_feature 1..119: note = Description of Artificial Sequence: Artificial DNA
  source 1..119: mol_type = other DNA
aagaaggagatatacatatggttaaaaaaacaaaaacannntgtnnnnnnnnnnnnnnnnnnnnnnnnnnnnnnnnnnnnnnnnnnnnnnnnnnntagnnnggcggttctggcggtagc

SEQ ID NO: 16 - DNA, 122 bp, synthetic construct
  misc_feature 1..122: note = Description of Artificial Sequence: Artificial DNA
  source 1..122: mol_type = other DNA
aagaaggagatatacatatggttaaaaaaacaaaaacannntgtnnnnnnnnnnnnnnnnnnnnnnnnnnnnnnnnnnnnnnnnnnnnnnnnnnnnnntagnnnggcggttctggcggtagc

SEQ ID NO: 17 - RNA, 23 nt, synthetic construct
  misc_feature 1..23: note = Description of Artificial Sequence: Artificial RNA
  source 1..23: mol_type = other RNA
taccccccgccgccccccgtcct

SEQ ID NO: 18 - DNA, 123 bp, synthetic construct
  misc_feature 1..123: note = Description of Artificial Sequence: Artificial DNA
  source 1..123: mol_type = other DNA
gttgtaaaacgacggccagtgccaagcttgggctaatacgactcactatagggagagtagttcaatggtagaacgtcggtctctaaaaccgagcgttgagggttcgattcctttctctcccac

SEQ ID NO: 19 - DNA, 18 bp, synthetic construct
  misc_feature 1..18: note = Description of Artificial Sequence: Artificial DNA
  source 1..18: mol_type = other DNA
gctaccgccagaaccacc

SEQ ID NO: 20 - DNA, 32 bp, synthetic construct
  misc_feature 1..32: note = Description of Artificial Sequence: Artificial DNA
  source 1..32: mol_type = other DNA
ggagatatacatatggttaagaaaacaaaaac

SEQ ID NO: 21 - DNA, 20 bp, synthetic construct
  misc_feature 1..20: note = Description of Artificial Sequence: Artificial DNA
  source 1..20: mol_type = other DNA
ctgctaccgccagaaccacc

SEQ ID NO: 22 - protein, 6 aa, synthetic construct
  REGION 1..6: note = Description of Artificial Sequence: Artificial peptide
VKKTKT

SEQ ID NO: 23 - protein, 10 aa, synthetic construct
  REGION 1..10: note = Description of Artificial Sequence: Artificial peptide
EQKLISEEDL

SEQ ID NO: 24 - protein, 11 aa, synthetic construct
  REGION 1..11: note = Description of Artificial Sequence: Artificial peptide
VSGWRLFKKIS

SEQ ID NO: 25 - protein, 57 aa, synthetic construct
  REGION 1..57: note = Description of Artificial Sequence: Artificial peptide
MVKKTKTHCSYERLQFHGHEAPFRVXVGSGSGSEQKLISEEDLGGSVSGWRLFKKIS

SEQ ID NO: 26 - DNA, 273 bp, synthetic construct
  misc_feature 1..273: note = Description of Artificial Sequence: Artificial DNA
  source 1..273: mol_type = other DNA
gaaattaatacgactcactatagggagaccacaacggtttccctctagaaataattttgtttaactttaagaaggagatataccaatggttaaaaaaacaaaaacacattgctcttacgaacgtctgcagttccatggtcatgaagctccgttccgtgtttaggttggttctggcagtggttccgaacagaaactgatcagcgaagaagatctgggtggctctgtaagtggatggcgattattcaagaagattagctaatgaataactaatcc

SEQ ID NO: 27 - DNA, 24 bp, synthetic construct
  misc_feature 1..24: note = Description of Artificial Sequence: Artificial DNA
  source 1..24: mol_type = other DNA
gaaattaatacgactcactatagg

SEQ ID NO: 28 - DNA, 17 bp, synthetic construct
  misc_feature 1..17: note = Description of Artificial Sequence: Artificial DNA
  source 1..17: mol_type = other DNA
gaaccactgccagaacc

SEQ ID NO: 29 - DNA, 105 bp, synthetic construct
  misc_feature 1..105: note = Description of Artificial Sequence: Artificial DNA
  source 1..105: mol_type = other DNA
gaaattaatacgactcactatagggagaccacaacggtttccctctagaaataattttgtttaactttaagaaggagatataccaatggttaaaaaaacaaaaac

SEQ ID NO: 30 - DNA, 95 bp, synthetic construct
  misc_feature 1..95: note = Description of Artificial Sequence: Artificial DNA
  source 1..95: mol_type = other DNA
gaaccactgccagaaccaacctaaacacggaacggagcttcatgaccatggaactgcagacgttcgtaagagcaatgtgtttttgtttttttaac

SEQ ID NO: 31 - DNA, 24 bp, synthetic construct
  misc_feature 1..24: note = Description of Artificial Sequence: Artificial DNA
  source 1..24: mol_type = other DNA
ggattagttattcattagctaatc

SEQ ID NO: 32 - DNA, 107 bp, synthetic construct
  misc_feature 1..107: note = Description of Artificial Sequence: Artificial DNA
  source 1..107: mol_type = other DNA
ggttctggcagtggttccgaacagaaactgatcagcgaagaagatctgggtggctctgtaagtggatggcgattattcaagaagattagctaatgaataactaatcc

SEQ ID NO: 33 - protein, 24 aa, synthetic construct
  REGION 1..24: note = Description of Artificial Sequence: Artificial peptide
EQKLISEEDLGGSVSGWRLFKKIS

SEQ ID NO: 34 - protein, 15 aa, synthetic construct
  REGION 1..15: note = Description of Artificial Sequence: Cyclic peptide
CRALLRGAPFHLAEC

SEQ ID NO: 35 - protein, 12 aa, synthetic construct
  REGION 1..12: note = Description of Artificial Sequence: Cyclic peptide
CDRTLLYYRLSC

SEQ ID NO: 36 - protein, 15 aa, synthetic construct
  REGION 1..15: note = Description of Artificial Sequence: Cyclic peptide
CRALLRGAPFHLAEK

SEQ ID NO: 37 - protein, 12 aa, synthetic construct
  REGION 1..12: note = Description of Artificial Sequence: Cyclic peptide
CDRTLLYYRLSK

SEQ ID NO: 38 - protein, 20 aa, synthetic construct
  REGION 1..20: note = Description of Artificial Sequence: Cyclic peptide
ICVYTFDAHAHSLHAALTKI

SEQ ID NO: 39 - protein, 20 aa, synthetic construct
  REGION 1..20: note = Description of Artificial Sequence: Cyclic peptide
ACVYTFDAHAHSLHAALTKI

SEQ ID NO: 40 - protein, 20 aa, synthetic construct
  REGION 1..20: note = Description of Artificial Sequence: Cyclic peptide
GCVYTFDAHAHSLHAALTKI

SEQ ID NO: 41 - protein, 20 aa, synthetic construct
  REGION 1..20: note = Description of Artificial Sequence: Cyclic peptide
PCVYTFDAHAHSLHAALTKI

SEQ ID NO: 42 - protein, 20 aa, synthetic construct
  REGION 1..20: note = Description of Artificial Sequence: Cyclic peptide
LCVYTFDAHAHSLHAALTKI

SEQ ID NO: 43 - protein, 20 aa, synthetic construct
  REGION 1..20: note = Description of Artificial Sequence: Cyclic peptide
VCVYTFDAHAHSLHAALTKI

SEQ ID NO: 44 - protein, 20 aa, synthetic construct
  REGION 1..20: note = Description of Artificial Sequence: Cyclic peptide
FCVYTFDAHAHSLHAALTKI

SEQ ID NO: 45 - protein, 20 aa, synthetic construct
  REGION 1..20: note = Description of Artificial Sequence: Cyclic peptide
YCVYTFDAHAHSLHAALTKI

SEQ ID NO: 46 - protein, 20 aa, synthetic construct
  REGION 1..20: note = Description of Artificial Sequence: Cyclic peptide
WCVYTFDAHAHSLHAALTKI

SEQ ID NO: 47 - protein, 20 aa, synthetic construct
  REGION 1..20: note = Description of Artificial Sequence: Cyclic peptide
NCVYTFDAHAHSLHAALTKI

SEQ ID NO: 48 - protein, 20 aa, synthetic construct
  REGION 1..20: note = Description of Artificial Sequence: Cyclic peptide
QCVYTFDAHAHSLHAALTKI

SEQ ID NO: 49 - protein, 20 aa, synthetic construct
  REGION 1..20: note = Description of Artificial Sequence: Cyclic peptide
SCVYTFDAHAHSLHAALTKI

SEQ ID NO: 50 - protein, 20 aa, synthetic construct
  REGION 1..20: note = Description of Artificial Sequence: Cyclic peptide
TCVYTFDAHAHSLHAALTKI

SEQ ID NO: 51 - protein, 20 aa, synthetic construct
  REGION 1..20: note = Description of Artificial Sequence: Cyclic peptide
DCVYTFDAHAHSLHAALTKI

SEQ ID NO: 52 - protein, 20 aa, synthetic construct
  REGION 1..20: note = Description of Artificial Sequence: Cyclic peptide
ECVYTFDAHAHSLHAALTKI

SEQ ID NO: 53 - protein, 20 aa, synthetic construct
  REGION 1..20: note = Description of Artificial Sequence: Cyclic peptide
RCVYTFDAHAHSLHAALTKI

SEQ ID NO: 54 - protein, 20 aa, synthetic construct
  REGION 1..20: note = Description of Artificial Sequence: Cyclic peptide
HCVYTFDAHAHSLHAALTKI

SEQ ID NO: 55 - protein, 20 aa, synthetic construct
  REGION 1..20: note = Description of Artificial Sequence: Cyclic peptide
ICAYTFDAHAHSLHAALTKI

SEQ ID NO: 56 - protein, 20 aa, synthetic construct
  REGION 1..20: note = Description of Artificial Sequence: Cyclic peptide
ICLYTFDAHAHSLHAALTKI

SEQ ID NO: 57 - protein, 20 aa, synthetic construct
  REGION 1..20: note = Description of Artificial Sequence: Cyclic peptide
ICIYTFDAHAHSLHAALTKI

SEQ ID NO: 58 - protein, 20 aa, synthetic construct
  REGION 1..20: note = Description of Artificial Sequence: Cyclic peptide
ICFYTFDAHAHSLHAALTKI

SEQ ID NO: 59 - protein, 20 aa, synthetic construct
  REGION 1..20: note = Description of Artificial Sequence: Cyclic peptide
ICYYTFDAHAHSLHAALTKI

SEQ ID NO: 60 - protein, 20 aa, synthetic construct
  REGION 1..20: note = Description of Artificial Sequence: Cyclic peptide
ICTYTFDAHAHSLHAALTKI

SEQ ID NO: 61 - protein, 20 aa, synthetic construct
  REGION 1..20: note = Description of Artificial Sequence: Cyclic peptide
ICVFTFDAHAHSLHAALTKI

SEQ ID NO: 62 - protein, 20 aa, synthetic construct
  REGION 1..20: note = Description of Artificial Sequence: Cyclic peptide
ICVWTFDAHAHSLHAALTKI

SEQ ID NO: 63 - protein, 20 aa, synthetic construct
  REGION 1..20: note = Description of Artificial Sequence: Cyclic peptide
ICVHTFDAHAHSLHAALTKI

SEQ ID NO: 64 - protein, 20 aa, synthetic construct
  REGION 1..20: note = Description of Artificial Sequence: Cyclic peptide
ICVYAFDAHAHSLHAALTKI

SEQ ID NO: 65 - protein, 20 aa, synthetic construct
  REGION 1..20: note = Description of Artificial Sequence: Cyclic peptide
ICVYGFDAHAHSLHAALTKI

SEQ ID NO: 66 - protein, 20 aa, synthetic construct
  REGION 1..20: note = Description of Artificial Sequence: Cyclic peptide
ICVYLFDAHAHSLHAALTKI

SEQ ID NO: 67 - protein, 20 aa, synthetic construct
  REGION 1..20: note = Description of Artificial Sequence: Cyclic peptide
ICVYIFDAHAHSLHAALTKI

SEQ ID NO: 68 - protein, 20 aa, synthetic construct
  REGION 1..20: note = Description of Artificial Sequence: Cyclic peptide
ICVYVFDAHAHSLHAALTKI

SEQ ID NO: 69 - protein, 20 aa, synthetic construct
  REGION 1..20: note = Description of Artificial Sequence: Cyclic peptide
ICVYQFDAHAHSLHAALTKI

SEQ ID NO: 70 - protein, 20 aa, synthetic construct
  REGION 1..20: note = Description of Artificial Sequence: Cyclic peptide
ICVYSFDAHAHSLHAALTKI

SEQ ID NO: 71 - protein, 20 aa, synthetic construct
  REGION 1..20: note = Description of Artificial Sequence: Cyclic peptide
ICVYEFDAHAHSLHAALTKI

SEQ ID NO: 72 - protein, 20 aa, synthetic construct
  REGION 1..20: note = Description of Artificial Sequence: Cyclic peptide
ICVYRFDAHAHSLHAALTKI

SEQ ID NO: 73 - protein, 20 aa, synthetic construct
  REGION 1..20: note = Description of Artificial Sequence: Cyclic peptide
ICVYHFDAHAHSLHAALTKI

SEQ ID NO: 74 - protein, 20 aa, synthetic construct
  REGION 1..20: note = Description of Artificial Sequence: Cyclic peptide
ICVYTADAHAHSLHAALTKI

SEQ ID NO: 75 - protein, 20 aa, synthetic construct
  REGION 1..20: note = Description of Artificial Sequence: Cyclic peptide
ICVYTGDAHAHSLHAALTKI

SEQ ID NO: 76 - protein, 20 aa, synthetic construct
  REGION 1..20: note = Description of Artificial Sequence: Cyclic peptide
ICVYTYDAHAHSLHAALTKI

SEQ ID NO: 77 - protein, 20 aa, synthetic construct
  REGION 1..20: note = Description of Artificial Sequence: Cyclic peptide
ICVYTWDAHAHSLHAALTKI

SEQ ID NO: 78 - protein, 20 aa, synthetic construct
  REGION 1..20: note = Description of Artificial Sequence: Cyclic peptide
ICVYTSDAHAHSLHAALTKI

SEQ ID NO: 79 - protein, 20 aa, synthetic construct
  REGION 1..20: note = Description of Artificial Sequence: Cyclic peptide
ICVYTHDAHAHSLHAALTKI

SEQ ID NO: 80 - protein, 20 aa, synthetic construct
  REGION 1..20: note = Description of Artificial Sequence: Cyclic peptide
ICVYTFAAHAHSLHAALTKI

SEQ ID NO: 81 - protein, 20 aa, synthetic construct
  REGION 1..20: note = Description of Artificial Sequence: Cyclic peptide
ICVYTFGAHAHSLHAALTKI

SEQ ID NO: 82 - protein, 20 aa, synthetic construct
  REGION 1..20: note = Description of Artificial Sequence: Cyclic peptide
ICVYTFPAHAHSLHAALTKI

SEQ ID NO: 83 - protein, 20 aa, synthetic construct
  REGION 1..20: note = Description of Artificial Sequence: Cyclic peptide
ICVYTFVAHAHSLHAALTKI

SEQ ID NO: 84 - protein, 20 aa, synthetic construct
  REGION 1..20: note = Description of Artificial Sequence: Cyclic peptide
ICVYTFFAHAHSLHAALTKI

SEQ ID NO: 85 - protein, 20 aa, synthetic construct
  REGION 1..20: note = Description of Artificial Sequence: Cyclic peptide
ICVYTFYAHAHSLHAALTKI

SEQ ID NO: 86 - protein, 20 aa, synthetic construct
  REGION 1..20: note = Description of Artificial Sequence: Cyclic peptide
ICVYTFWAHAHSLHAALTKI

SEQ ID NO: 87 - protein, 20 aa, synthetic construct
  REGION 1..20: note = Description of Artificial Sequence: Cyclic peptide
ICVYTFNAHAHSLHAALTKI

SEQ ID NO: 88 - protein, 20 aa, synthetic construct
  REGION 1..20: note = Description of Artificial Sequence: Cyclic peptide
ICVYTFSAHAHSLHAALTKI

SEQ ID NO: 89 - protein, 20 aa, synthetic construct
  REGION 1..20: note = Description of Artificial Sequence: Cyclic peptide
ICVYTFDGHAHSLHAALTKI

SEQ ID NO: 90 - protein, 20 aa, synthetic construct
  REGION 1..20: note = Description of Artificial Sequence: Cyclic peptide
ICVYTFDPHAHSLHAALTKI

SEQ ID NO: 91 - protein, 20 aa, synthetic construct
  REGION 1..20: note = Description of Artificial Sequence: Cyclic peptide
ICVYTFDLHAHSLHAALTKI

SEQ ID NO: 92 - protein, 20 aa, synthetic construct
  REGION 1..20: note = Description of Artificial Sequence: Cyclic peptide
ICVYTFDIHAHSLHAALTKI

SEQ ID NO: 93 - protein, 20 aa, synthetic construct
  REGION 1..20: note = Description of Artificial Sequence: Cyclic peptide
ICVYTFDVHAHSLHAALTKI

SEQ ID NO: 94 - protein, 20 aa, synthetic construct
  REGION 1..20: note = Description of Artificial Sequence: Cyclic peptide
ICVYTFDYHAHSLHAALTKI

SEQ ID NO: 95 - protein, 20 aa, synthetic construct
  REGION 1..20: note = Description of Artificial Sequence: Cyclic peptide
ICVYTFDWHAHSLHAALTKI

SEQ ID NO: 96 - protein, 20 aa, synthetic construct
  REGION 1..20: note = Description of Artificial Sequence: Cyclic peptide
ICVYTFDNHAHSLHAALTKI

SEQ ID NO: 97 - protein, 20 aa, synthetic construct
  REGION 1..20: note = Description of Artificial Sequence: Cyclic peptide
ICVYTFDQHAHSLHAALTKI

SEQ ID NO: 98 - protein, 20 aa, synthetic construct
  REGION 1..20: note = Description of Artificial Sequence: Cyclic peptide
ICVYTFDSHAHSLHAALTKI

SEQ ID NO: 99 - protein, 20 aa, synthetic construct
  REGION 1..20: note = Description of Artificial Sequence: Cyclic peptide
ICVYTFDTHAHSLHAALTKI

SEQ ID NO: 100 - protein, 20 aa, synthetic construct
  REGION 1..20: note = Description of Artificial Sequence: Cyclic peptide
ICVYTFDEHAHSLHAALTKI

SEQ ID NO: 101 - protein, 20 aa, synthetic construct
  REGION 1..20: note = Description of Artificial Sequence: Cyclic peptide
ICVYTFDRHAHSLHAALTKI

SEQ ID NO: 102 - protein, 20 aa, synthetic construct
  REGION 1..20: note = Description of Artificial Sequence: Cyclic peptide
ICVYTFDHHAHSLHAALTKI

SEQ ID NO: 103 - protein, 20 aa, synthetic construct
  REGION 1..20: note = Description of Artificial Sequence: Cyclic peptide
ICVYTFDAAAHSLHAALTKI

SEQ ID NO: 104 - protein, 20 aa, synthetic construct
  REGION 1..20: note = Description of Artificial Sequence: Cyclic peptide
ICVYTFDAGAHSLHAALTKI

SEQ ID NO: 105 - protein, 20 aa, synthetic construct
  REGION 1..20: note = Description of Artificial Sequence: Cyclic peptide
ICVYTFDALAHSLHAALTKI

SEQ ID NO: 106 - protein, 20 aa, synthetic construct
  REGION 1..20: note = Description of Artificial Sequence: Cyclic peptide
ICVYTFDAIAHSLHAALTKI

SEQ ID NO: 107 - protein, 20 aa, synthetic construct
  REGION 1..20: note = Description of Artificial Sequence: Cyclic peptide
ICVYTFDAVAHSLHAALTKI

SEQ ID NO: 108 - protein, 20 aa, synthetic construct
  REGION 1..20: note = Description of Artificial Sequence: Cyclic peptide
ICVYTFDAFAHSLHAALTKI

SEQ ID NO: 109 - protein, 20 aa, synthetic construct
  REGION 1..20: note = Description of Artificial Sequence: Cyclic peptide
ICVYTFDAYAHSLHAALTKI

SEQ ID NO: 110 - protein, 20 aa, synthetic construct
  REGION 1..20: note = Description of Artificial Sequence: Cyclic peptide
ICVYTFDAWAHSLHAALTKI

SEQ ID NO: 111 - protein, 20 aa, synthetic construct
  REGION 1..20: note = Description of Artificial Sequence: Cyclic peptide
ICVYTFDANAHSLHAALTKI

SEQ ID NO: 112 - protein, 20 aa, synthetic construct
  REGION 1..20: note = Description of Artificial Sequence: Cyclic peptide
ICVYTFDAQAHSLHAALTKI

SEQ ID NO: 113 - protein, 20 aa, synthetic construct
  REGION 1..20: note = Description of Artificial Sequence: Cyclic peptide
ICVYTFDASAHSLHAALTKI

SEQ ID NO: 114 - protein, 20 aa, synthetic construct
  REGION 1..20: note = Description of Artificial Sequence: Cyclic peptide
ICVYTFDATAHSLHAALTKI

SEQ ID NO: 115 - protein, 20 aa, synthetic construct
  REGION 1..20: note = Description of Artificial Sequence: Cyclic peptide
ICVYTFDADAHSLHAALTKI

SEQ ID NO: 116 - protein, 20 aa, synthetic construct
  REGION 1..20: note = Description of Artificial Sequence: Cyclic peptide
ICVYTFDAEAHSLHAALTKI

SEQ ID NO: 117 - protein, 20 aa, synthetic construct
  REGION 1..20: note = Description of Artificial Sequence: Cyclic peptide
ICVYTFDARAHSLHAALTKI

SEQ ID NO: 118 - protein, 20 aa, synthetic construct
  REGION 1..20: note = Description of Artificial Sequence: Cyclic peptide
ICVYTFDAHGHSLHAALTKI

SEQ ID NO: 119 - protein, 20 aa, synthetic construct
  REGION 1..20: note = Description of Artificial Sequence: Cyclic peptide
ICVYTFDAHIHSLHAALTKI

SEQ ID NO: 120 - protein, 20 aa, synthetic construct
  REGION 1..20: note = Description of Artificial Sequence: Cyclic peptide
ICVYTFDAHVHSLHAALTKI

SEQ ID NO: 121 - protein, 20 aa, synthetic construct
  REGION 1..20: note = Description of Artificial Sequence: Cyclic peptide
ICVYTFDAHFHSLHAALTKI

SEQ ID NO: 122 - protein, 20 aa, synthetic construct
  REGION 1..20: note = Description of Artificial Sequence: Cyclic peptide
ICVYTFDAHYHSLHAALTKI

SEQ ID NO: 123 - protein, 20 aa, synthetic construct
  REGION 1..20: note = Description of Artificial Sequence: Cyclic peptide
ICVYTFDAHWHSLHAALTKI

SEQ ID NO: 124 - protein, 20 aa, synthetic construct
  REGION 1..20: note = Description of Artificial Sequence: Cyclic peptide
ICVYTFDAHQHSLHAALTKI

SEQ ID NO: 125 - protein, 20 aa, synthetic construct
  REGION 1..20: note = Description of Artificial Sequence: Cyclic peptide
ICVYTFDAHSHSLHAALTKI

SEQ ID NO: 126 - protein, 20 aa, synthetic construct
  REGION 1..20: note = Description of Artificial Sequence: Cyclic peptide
ICVYTFDAHTHSLHAALTKI

SEQ ID NO: 127 - protein, 20 aa, synthetic construct
  REGION 1..20: note = Description of Artificial Sequence: Cyclic peptide
ICVYTFDAHDHSLHAALTKI

SEQ ID NO: 128 - protein, 20 aa, synthetic construct
  REGION 1..20: note = Description of Artificial Sequence: Cyclic peptide
ICVYTFDAHEHSLHAALTKI

SEQ ID NO: 129 - protein, 20 aa, synthetic construct
  REGION 1..20: note = Description of Artificial Sequence: Cyclic peptide
ICVYTFDAHRHSLHAALTKI

SEQ ID NO: 130 - protein, 20 aa, synthetic construct
  REGION 1..20: note = Description of Artificial Sequence: Cyclic peptide
ICVYTFDAHHHSLHAALTKI

SEQ ID NO: 131 - protein, 20 aa, synthetic construct
  REGION 1..20: note = Description of Artificial Sequence: Cyclic peptide
ICVYTFDAHAASLHAALTKI

SEQ ID NO: 132 - protein, 20 aa, synthetic construct
  REGION 1..20: note = Description of Artificial Sequence: Cyclic peptide
ICVYTFDAHAGSLHAALTKI

SEQ ID NO: 133 - protein, 20 aa, synthetic construct
  REGION 1..20: note = Description of Artificial Sequence: Cyclic peptide
ICVYTFDAHAPSLHAALTKI

SEQ ID NO: 134 - protein, 20 aa, synthetic construct
  REGION 1..20: note = Description of Artificial Sequence: Cyclic peptide
ICVYTFDAHALSLHAALTKI

SEQ ID NO: 135 - protein, 20 aa, synthetic construct
  REGION 1..20: note = Description of Artificial Sequence: Cyclic peptide
ICVYTFDAHAISLHAALTKI

SEQ ID NO: 136 - protein, 20 aa, synthetic construct
  REGION 1..20: note = Description of Artificial Sequence: Cyclic peptide
ICVYTFDAHAVSLHAALTKI

SEQ ID NO: 137 - protein, 20 aa, synthetic construct
  REGION 1..20: note = Description of Artificial Sequence: Cyclic peptide
ICVYTFDAHAFSLHAALTKI

SEQ ID NO: 138 - protein, 20 aa, synthetic construct
  REGION 1..20: note = Description of Artificial Sequence: Cyclic peptide
ICVYTFDAHAYSLHAALTKI

SEQ ID NO: 139 - protein, 20 aa, synthetic construct
  REGION 1..20: note = Description of Artificial Sequence: Cyclic peptide
ICVYTFDAHAWSLHAALTKI

SEQ ID NO: 140 - protein, 20 aa, synthetic construct
  REGION 1..20: note = Description of Artificial Sequence: Cyclic peptide
ICVYTFDAHANSLHAALTKI

SEQ ID NO: 141 - protein, 20 aa, synthetic construct
  REGION 1..20: note = Description of Artificial Sequence: Cyclic peptide
ICVYTFDAHAQSLHAALTKI

SEQ ID NO: 142 - protein, 20 aa, synthetic construct
  REGION 1..20: note = Description of Artificial Sequence: Cyclic peptide
ICVYTFDAHASSLHAALTKI

SEQ ID NO: 143 - protein, 20 aa, synthetic construct
  REGION 1..20: note = Description of Artificial Sequence: Cyclic peptide
ICVYTFDAHATSLHAALTKI

SEQ ID NO: 144 - protein, 20 aa, synthetic construct
  REGION 1..20: note = Description of Artificial Sequence: Cyclic peptide
ICVYTFDAHADSLHAALTKI

SEQ ID NO: 145 - protein, 20 aa, synthetic construct
  REGION 1..20: note = Description of Artificial Sequence: Cyclic peptide
ICVYTFDAHAESLHAALTKI

SEQ ID NO: 146 - protein, 20 aa, synthetic construct
  REGION 1..20: note = Description of Artificial Sequence: Cyclic peptide
ICVYTFDAHARSLHAALTKI

SEQ ID NO: 147 - protein, 20 aa, synthetic construct
  REGION 1..20: note = Description of Artificial Sequence: Cyclic peptide
ICVYTFDAHAHALHAALTKI

SEQ ID NO: 148 - protein, 20 aa, synthetic construct
  REGION 1..20: note = Description of Artificial Sequence: Cyclic peptide
ICVYTFDAHAHGLHAALTKI

SEQ ID NO: 149 - protein, 20 aa, synthetic construct
  REGION 1..20: note = Description of Artificial Sequence: Cyclic peptide
ICVYTFDAHAHLLHAALTKI

SEQ ID NO: 150 - protein, 20 aa, synthetic construct
  REGION 1..20: note = Description of Artificial Sequence: Cyclic peptide
ICVYTFDAHAHILHAALTKI

SEQ ID NO: 151 - protein, 20 aa, synthetic construct
  REGION 1..20: note = Description of Artificial Sequence: Cyclic peptide
ICVYTFDAHAHVLHAALTKI

SEQ ID NO: 152 - protein, 20 aa, synthetic construct
  REGION 1..20: note = Description of Artificial Sequence: Cyclic peptide
ICVYTFDAHAHFLHAALTKI

SEQ ID NO: 153 - protein, 20 aa, synthetic construct
  REGION 1..20: note = Description of Artificial Sequence: Cyclic peptide
ICVYTFDAHAHYLHAALTKI

SEQ ID NO: 154 - protein, 20 aa, synthetic construct
  REGION 1..20: note = Description of Artificial Sequence: Cyclic peptide
ICVYTFDAHAHWLHAALTKI

SEQ ID NO: 155 - protein, 20 aa, synthetic construct
  REGION 1..20: note = Description of Artificial Sequence: Cyclic peptide
ICVYTFDAHAHNLHAALTKI

SEQ ID NO: 156 - protein, 20 aa, synthetic construct
  REGION 1..20: note = Description of Artificial Sequence: Cyclic peptide
ICVYTFDAHAHQLHAALTKI

SEQ ID NO: 157 - protein, 20 aa, synthetic construct
  REGION 1..20: note = Description of Artificial Sequence: Cyclic peptide
ICVYTFDAHAHTLHAALTKI

SEQ ID NO: 158 - protein, 20 aa, synthetic construct
  REGION 1..20: note = Description of Artificial Sequence: Cyclic peptide
ICVYTFDAHAHDLHAALTKI

SEQ ID NO: 159 - protein, 20 aa, synthetic construct
  REGION 1..20: note = Description of Artificial Sequence: Cyclic peptide
ICVYTFDAHAHELHAALTKI

SEQ ID NO: 160 - protein, 20 aa, synthetic construct
  REGION 1..20: note = Description of Artificial Sequence: Cyclic peptide
ICVYTFDAHAHRLHAALTKI

SEQ ID NO: 161 - protein, 20 aa, synthetic construct
  REGION 1..20: note = Description of Artificial Sequence: Cyclic peptide
ICVYTFDAHAHHLHAALTKI

SEQ ID NO: 162 - protein, 20 aa, synthetic construct
  REGION 1..20: note = Description of Artificial Sequence: Cyclic peptide
ICVYTFDAHAHSAHAALTKI

SEQ ID NO: 163 - protein, 20 aa, synthetic construct
  REGION 1..20: note = Description of Artificial Sequence: Cyclic peptide
ICVYTFDAHAHSGHAALTKI

SEQ ID NO: 164 - protein, 20 aa, synthetic construct
  REGION 1..20: note = Description of Artificial Sequence: Cyclic peptide
ICVYTFDAHAHSPHAALTKI

SEQ ID NO: 165 - protein, 20 aa, synthetic construct
  REGION 1..20: note = Description of Artificial Sequence: Cyclic peptide
ICVYTFDAHAHSIHAALTKI

SEQ ID NO: 166 - protein, 20 aa, synthetic construct
  REGION 1..20: note = Description of Artificial Sequence: Cyclic peptide
ICVYTFDAHAHSVHAALTKI

SEQ ID NO: 167 - protein, 20 aa, synthetic construct
  REGION 1..20: note = Description of Artificial Sequence: Cyclic peptide
ICVYTFDAHAHSFHAALTKI

SEQ ID NO: 168 - protein, 20 aa, synthetic construct
  REGION 1..20: note = Description of Artificial Sequence: Cyclic peptide
ICVYTFDAHAHSYHAALTKI

SEQ ID NO: 169 - protein, 20 aa, synthetic construct
  REGION 1..20: note = Description of Artificial Sequence: Cyclic peptide
ICVYTFDAHAHSWHAALTKI

SEQ ID NO: 170 - protein, 20 aa, synthetic construct
  REGION 1..20: note = Description of Artificial Sequence: Cyclic peptide
ICVYTFDAHAHSQHAALTKI

SEQ ID NO: 171 - protein, 20 aa, synthetic construct
  REGION 1..20: note = Description of Artificial Sequence: Cyclic peptide
ICVYTFDAHAHSSHAALTKI

SEQ ID NO: 172 - protein, 20 aa, synthetic construct
  REGION 1..20: note = Description of Artificial Sequence: Cyclic peptide
ICVYTFDAHAHSTHAALTKI

SEQ ID NO: 173 - protein, 20 aa, synthetic construct
  REGION 1..20: note = Description of Artificial Sequence: Cyclic peptide
ICVYTFDAHAHSEHAALTKI

SEQ ID NO: 174 - protein, 20 aa, synthetic construct
  REGION 1..20: note = Description of Artificial Sequence: Cyclic peptide
ICVYTFDAHAHSRHAALTKI

SEQ ID NO: 175 - protein, 20 aa, synthetic construct
  REGION 1..20: note = Description of Artificial Sequence: Cyclic peptide
ICVYTFDAHAHSHHAALTKI

SEQ ID NO: 176 - protein, 20 aa, synthetic construct
  REGION 1..20: note = Description of Artificial Sequence: Cyclic peptide
ICVYTFDAHAHSLAAALTKI

SEQ ID NO: 177 - protein, 20 aa, synthetic construct
  REGION 1..20: note = Description of Artificial Sequence: Cyclic peptide
ICVYTFDAHAHSLGAALTKI

SEQ ID NO: 178 - protein, 20 aa, synthetic construct
  REGION 1..20: note = Description of Artificial Sequence: Cyclic peptide
ICVYTFDAHAHSLPAALTKI

SEQ ID NO: 179 - protein, 20 aa, synthetic construct
  REGION 1..20: note = Description of Artificial Sequence: Cyclic peptide
ICVYTFDAHAHSLLAALTKI

SEQ ID NO: 180 - protein, 20 aa, synthetic construct
  REGION 1..20: note = Description of Artificial Sequence: Cyclic peptide
ICVYTFDAHAHSLIAALTKI

SEQ ID NO: 181 - protein, 20 aa, synthetic construct
  REGION 1..20: note = Description of Artificial Sequence: Cyclic peptide
ICVYTFDAHAHSLVAALTKI

SEQ ID NO: 182 - protein, 20 aa, synthetic construct
  REGION 1..20: note = Description of Artificial Sequence: Cyclic peptide
ICVYTFDAHAHSLFAALTKI

SEQ ID NO: 183 - protein, 20 aa, synthetic construct
  REGION 1..20: note = Description of Artificial Sequence: Cyclic peptide
ICVYTFDAHAHSLYAALTKI

SEQ ID NO: 184 - protein, 20 aa, synthetic construct
  REGION 1..20: note = Description of Artificial Sequence: Cyclic peptide
ICVYTFDAHAHSLWAALTKI

SEQ ID NO: 185 - protein, 20 aa, synthetic construct
  REGION 1..20: note = Description of Artificial Sequence: Cyclic peptide
ICVYTFDAHAHSLNAALTKI

SEQ ID NO: 186 - protein, 20 aa, synthetic construct
  REGION 1..20: note = Description of Artificial Sequence: Cyclic peptide
ICVYTFDAHAHSLQAALTKI

SEQ ID NO: 187 - protein, 20 aa, synthetic construct
  REGION 1..20: note = Description of Artificial Sequence: Cyclic peptide
ICVYTFDAHAHSLSAALTKI

SEQ ID NO: 188 - protein, 20 aa, synthetic construct
  REGION 1..20: note = Description of Artificial Sequence: Cyclic peptide
ICVYTFDAHAHSLTAALTKI

SEQ ID NO: 189 - protein, 20 aa, synthetic construct
  REGION 1..20: note = Description of Artificial Sequence: Cyclic peptide
ICVYTFDAHAHSLDAALTKI

SEQ ID NO: 190 - protein, 20 aa, synthetic construct
  REGION 1..20: note = Description of Artificial Sequence: Cyclic peptide
ICVYTFDAHAHSLEAALTKI

SEQ ID NO: 191 - protein, 20 aa, synthetic construct
  REGION 1..20: note = Description of Artificial Sequence: Cyclic peptide
ICVYTFDAHAHSLRAALTKI

SEQ ID NO: 192 - protein, 20 aa, synthetic construct
  REGION 1..20: note = Description of Artificial Sequence: Cyclic peptide
ICVYTFDAHAHSLHGALTKI

SEQ ID NO: 193 - protein, 20 aa, synthetic construct
  REGION 1..20: note = Description of Artificial Sequence: Cyclic peptide
ICVYTFDAHAHSLHLALTKI

SEQ ID NO: 194 - protein, 20 aa, synthetic construct
  REGION 1..20: note = Description of Artificial Sequence: Cyclic peptide
ICVYTFDAHAHSLHIALTKI

SEQ ID NO: 195 - protein, 20 aa, synthetic construct
  REGION 1..20: note = Description of Artificial Sequence: Cyclic peptide
ICVYTFDAHAHSLHVALTKI

SEQ ID NO: 196 - protein, 20 aa, synthetic construct
  REGION 1..20: note = Description of Artificial Sequence: Cyclic peptide
ICVYTFDAHAHSLHFALTKI

SEQ ID NO: 197 - protein, 20 aa, synthetic construct
  REGION 1..20: note = Description of Artificial Sequence: Cyclic peptide
ICVYTFDAHAHSLHYALTKI

SEQ ID NO: 198 - protein, 20 aa, synthetic construct
  REGION 1..20: note = Description of Artificial Sequence: Cyclic peptide
ICVYTFDAHAHSLHWALTKI

SEQ ID NO: 199 - protein, 20 aa, synthetic construct
  REGION 1..20: note = Description of Artificial Sequence: Cyclic peptide
ICVYTFDAHAHSLHNALTKI

SEQ ID NO: 200 - protein, 20 aa, synthetic construct
  REGION 1..20: note = Description of Artificial Sequence: Cyclic peptide
ICVYTFDAHAHSLHQALTKI

SEQ ID NO: 201 - protein, 20 aa, synthetic construct
  REGION 1..20: note = Description of Artificial Sequence: Cyclic peptide
ICVYTFDAHAHSLHSALTKI

SEQ ID NO: 202 - protein, 20 aa, synthetic construct
  REGION 1..20: note = Description of Artificial Sequence: Cyclic peptide
ICVYTFDAHAHSLHTALTKI

SEQ ID NO: 203 - protein, 20 aa, synthetic construct
  REGION 1..20: note = Description of Artificial Sequence: Cyclic peptide
ICVYTFDAHAHSLHDALTKI

SEQ ID NO: 204 - protein, 20 aa, synthetic construct
  REGION 1..20: note = Description of Artificial Sequence: Cyclic peptide
ICVYTFDAHAHSLHEALTKI

SEQ ID NO: 205 - protein, 20 aa, synthetic construct
  REGION 1..20: note = Description of Artificial Sequence: Cyclic peptide
ICVYTFDAHAHSLHRALTKI

SEQ ID NO: 206 - protein, 20 aa, synthetic construct
  REGION 1..20: note = Description of Artificial Sequence: Cyclic peptide
ICVYTFDAHAHSLHHALTKI

SEQ ID NO: 207 - protein, 20 aa, synthetic construct
  REGION 1..20: note = Description of Artificial Sequence: Cyclic peptide
ICVYTFDAHAHSLHAILTKI

SEQ ID NO: 208 - protein, 20 aa, synthetic construct
  REGION 1..20: note = Description of Artificial Sequence: Cyclic peptide
ICVYTFDAHAHSLHAVLTKI

SEQ ID NO: 209 - protein, 20 aa, synthetic construct
  REGION 1..20: note = Description of Artificial Sequence: Cyclic peptide
ICVYTFDAHAHSLHASLTKI

SEQ ID NO: 210 - protein, 20 aa, synthetic construct
  REGION 1..20: note = Description of Artificial Sequence: Cyclic peptide
ICVYTFDAHAHSLHAAITKI

SEQ ID NO: 211 - protein, 20 aa, synthetic construct
  REGION 1..20: note = Description of Artificial Sequence: Cyclic peptide
ICVYTFDAHAHSLHAAVTKI

SEQ ID NO: 212 - protein, 20 aa, synthetic construct
  REGION 1..20: note = Description of Artificial Sequence: Cyclic peptide
ICVYTFDAHAHSLHAAFTKI

SEQ ID NO: 213 - protein, 20 aa, synthetic construct
  REGION 1..20: note = Description of Artificial Sequence: Cyclic peptide
ICVYTFDAHAHSLHAATTKI

SEQ ID NO: 214 - protein, 20 aa, synthetic construct
  REGION 1..20: note = Description of Artificial Sequence: Cyclic peptide
ICVYTFDAHAHSLHAALAKI

SEQ ID NO: 215 - protein, 20 aa, synthetic construct
  REGION 1..20: note = Description of Artificial Sequence: Cyclic peptide
ICVYTFDAHAHSLHAALGKI

SEQ ID NO: 216 - protein, 20 aa, synthetic construct
  REGION 1..20: note = Description of Artificial Sequence: Cyclic peptide
ICVYTFDAHAHSLHAALPKI

SEQ ID NO: 217 - protein, 20 aa, synthetic construct
  REGION 1..20: note = Description of Artificial Sequence: Cyclic peptide
ICVYTFDAHAHSLHAALVKI

SEQ ID NO: 218 - protein, 20 aa, synthetic construct
  REGION 1..20: note = Description of Artificial Sequence: Cyclic peptide
ICVYTFDAHAHSLHAALFKI

SEQ ID NO: 219 - protein, 20 aa, synthetic construct
  REGION 1..20: note = Description of Artificial Sequence: Cyclic peptide
ICVYTFDAHAHSLHAALNKI

SEQ ID NO: 220 - protein, 20 aa, synthetic construct
  REGION 1..20: note = Description of Artificial Sequence: Cyclic peptide
ICVYTFDAHAHSLHAALQKI

SEQ ID NO: 221 - protein, 20 aa, synthetic construct
  REGION 1..20: note = Description of Artificial Sequence: Cyclic peptide
ICVYTFDAHAHSLHAALSKI

SEQ ID NO: 222 - protein, 20 aa, synthetic construct
  REGION 1..20: note = Description of Artificial Sequence: Cyclic peptide
ICVYTFDAHAHSLHAALEKI

SEQ ID NO: 223 - protein, 20 aa, synthetic construct
  REGION 1..20: note = Description of Artificial Sequence: Cyclic peptide
ICVYTFDAHAHSLHAALRKI

SEQ ID NO: 224 - protein, 20 aa, synthetic construct
  REGION 1..20: note = Description of Artificial Sequence: Cyclic peptide
ICVYTFDAHAHSLHAALHKI

SEQ ID NO: 225 - protein, 20 aa, synthetic construct
  REGION 1..20: note = Description of Artificial Sequence: Cyclic peptide
ICVYTFDAHAHSLHAALTKA

SEQ ID NO: 226 - protein, 20 aa, synthetic construct
  REGION 1..20: note = Description of Artificial Sequence: Cyclic peptide
ICVYTFDAHAHSLHAALTKL

SEQ ID NO: 227 - protein, 20 aa, synthetic construct
  REGION 1..20: note = Description of Artificial Sequence: Cyclic peptide
ICVYTFDAHAHSLHAALTKV

SEQ ID NO: 228 - protein, 20 aa, synthetic construct
  REGION 1..20: note = Description of Artificial Sequence: Cyclic peptide
ICVYTFDAHAHSLHAALTKF

SEQ ID NO: 229 - protein, 20 aa, synthetic construct
  REGION 1..20: note = Description of Artificial Sequence: Cyclic peptide
ICVYTFDAHAHSLHAALTKY

SEQ ID NO: 230 - protein, 20 aa, synthetic construct
  REGION 1..20: note = Description of Artificial Sequence: Cyclic peptide
ICVYTFDAHAHSLHAALTKW

SEQ ID NO: 231 - protein, 20 aa, synthetic construct
  REGION 1..20: note = Description of Artificial Sequence: Cyclic peptide
ICVYTFDAHAHSLHAALTKN

SEQ ID NO: 232 - protein, 20 aa, synthetic construct
  REGION 1..20: note = Description of Artificial Sequence: Cyclic peptide
ICVYTFDAHAHSLHAALTKQ

SEQ ID NO: 233 - protein, 20 aa, synthetic construct
  REGION 1..20: note = Description of Artificial Sequence: Cyclic peptide
ICVYTFDAHAHSLHAALTKS

SEQ ID NO: 234 - protein, 20 aa, synthetic construct
  REGION 1..20: note = Description of Artificial Sequence: Cyclic peptide
ICVYTFDAHAHSLHAALTKT

SEQ ID NO: 235 - protein, 20 aa, synthetic construct
  REGION 1..20: note = Description of Artificial Sequence: Cyclic peptide
ICVYTFDAHAHSLHAALTKR

SEQ ID NO: 236 - protein, 20 aa, synthetic construct
  REGION 1..20: note = Description of Artificial Sequence: Cyclic peptide
ICVYTFDAHAHSLHAALTKH

SEQ ID NO: 237 - protein, 20 aa, synthetic construct
  REGION 1..20: note = Description of Artificial Sequence: Cyclic peptide
VCIYTFNHLAQTYWQSLNKV

SEQ ID NO: 238 - protein, 20 aa, synthetic construct
  REGION 1..20: note = Description of Artificial Sequence: Cyclic peptide
VCIWVFNRFAHTLKESLTKV

SEQ ID NO: 239 - protein, 20 aa, synthetic construct
  REGION 1..20: note = Description of Artificial Sequence: Cyclic peptide
ACVWTFDRHAQEISQALHKV

SEQ ID NO: 240 - protein, 20 aa, synthetic construct
  REGION 1..20: note = Description of Artificial Sequence: Cyclic peptide
ACVYLFNWRATSYGKSLIKW

SEQ ID NO: 241 - protein, 21 aa, synthetic construct
  REGION 1..21: note = Description of Artificial Sequence: Cyclic peptide
HCKLYSYPLWYWPKWVFQTKE

SEQ ID NO: 242 - protein, 21 aa, synthetic construct
  REGION 1..21: note = Description of Artificial Sequence: Cyclic peptide
ACGVHQWEIGEWFGYRYYYKP

SEQ ID NO: 243 - protein, 21 aa, synthetic construct
  REGION 1..21: note = Description of Artificial Sequence: Cyclic peptide
QCYLPSWFYQKARLLFQYIKS

SEQ ID NO: 244 - protein, 21 aa, synthetic construct
  REGION 1..21: note = Description of Artificial Sequence: Cyclic peptide
DCTQGKILTYSQALFSFGVKI

SEQ ID NO: 245 - protein, 22 aa, synthetic construct
  REGION 1..22: note = Description of Artificial Sequence: Cyclic peptide
NCVYYAKPVFAHANRVWTYIKI

SEQ ID NO: 246 - protein, 22 aa, synthetic construct
  REGION 1..22: note = Description of Artificial Sequence: Cyclic peptide
PCIYTFDQSAIKYKIGFVLRKV

SEQ ID NO: 247 - protein, 22 aa, synthetic construct
  REGION 1..22: note = Description of Artificial Sequence: Cyclic peptide
PCQSYIWSHFIVVNRQWLHPKW

SEQ ID NO: 248 - protein, 22 aa, synthetic construct
  REGION 1..22: note = Description of Artificial Sequence: Cyclic peptide
QCWLQGPYWSDIKIYIYQHDKY

SEQ ID NO: 249 - protein, 22 aa, synthetic construct
  REGION 1..22: note = Description of Artificial Sequence: Cyclic peptide
VCVRPIFIFSFRAPFNAVDWKI

SEQ ID NO: 250 - protein, 20 aa, synthetic construct
  REGION 1..20: note = Description of Artificial Sequence: Cyclic peptide
QCIWQYLYQIASLFHVVGKA

SEQ ID NO: 251 - protein, 19 aa, synthetic construct
  REGION 1..19: note = Description of Artificial Sequence: Cyclic peptide
TCWTAWQWFGHWVPFVAKT

SEQ ID NO: 252 - protein, 18 aa, synthetic construct
  REGION 1..18: note = Description of Artificial Sequence: Cyclic peptide
RCVYSFDPARYPYHLKKV

SEQ ID NO: 253 - protein, 22 aa, synthetic construct
  REGION 1..22: note = Description of Artificial Sequence: Cyclic peptide
TCFSPGQIWIWTHLVTAIRNKT

SEQ ID NO: 254 - protein, 19 aa, synthetic construct
  REGION 1..19: note = Description of Artificial Sequence: Cyclic peptide
LCVYTFNWQQKFGHHLTKI

SEQ ID NO: 255 - protein, 21 aa, synthetic construct
  REGION 1..21: note = Description of Artificial Sequence: Cyclic peptide
FCTLWQFGNLVWTHESPFIKQ

SEQ ID NO: 256 - protein, 20 aa, synthetic construct
  REGION 1..20: note = Description of Artificial Sequence: Cyclic peptide
DCVYQYDRNAHYWDTALVKV

SEQ ID NO: 257 - protein, 21 aa, synthetic construct
  REGION 1..21: note = Description of Artificial Sequence: Cyclic peptide
FCAWVVDYQELHQFWSIVQKI

SEQ ID NO: 258 - protein, 22 aa, synthetic construct
  REGION 1..22: note = Description of Artificial Sequence: Cyclic peptide
VCVRPIFIFSFRAPFNAVDWKN

SEQ ID NO: 259 - protein, 21 aa, synthetic construct
  REGION 1..21: note = Description of Artificial Sequence: Cyclic peptide
TCNIWQFNPAARWGFHLVYKY

SEQ ID NO: 260 - protein, 22 aa, synthetic construct
  REGION 1..22: note = Description of Artificial Sequence: Cyclic peptide
ICREVIVGSLYTWDGNRGFFKV

SEQ ID NO: 261 - protein, 12 aa, synthetic construct
  REGION 1..12: note = Description of Artificial Sequence: Cyclic peptide
LCYINLFTHTKV

SEQ ID NO: 262 - protein, 13 aa, synthetic construct
  REGION 1..13: note = Description of Artificial Sequence: Cyclic peptide
WCNFANVWTFNKS

SEQ ID NO: 263 - protein, 13 aa, synthetic construct
  REGION 1..13: note = Description of Artificial Sequence: Cyclic peptide
QCYHIIVYTFVKP

SEQ ID NO: 264 - protein, 15 aa, synthetic construct
  REGION 1..15: note = Description of Artificial Sequence: Cyclic peptide
VCIFTWDRVHWPVKV

SEQ ID NO: 265 - protein, 15 aa, synthetic construct
  REGION 1..15: note = Description of Artificial Sequence: Cyclic peptide
VCIYTWDRQSWPVKL

SEQ ID NO: 266 - protein, 15 aa, synthetic construct
  REGION 1..15: note = Description of Artificial Sequence: Cyclic peptide
DCIWQWHPWSGYTKL

SEQ ID NO: 267 - protein, 15 aa, synthetic construct
  REGION 1..15: note = Description of Artificial Sequence: Cyclic peptide
DCIWQWTPTKSFQKL

SEQ ID NO: 268 - protein, 15 aa, synthetic construct
  REGION 1..15: note = Description of Artificial Sequence: Cyclic peptide
SCIYQWDYVHWPIKL

SEQ ID NO: 269 - protein, 15 aa, synthetic construct
  REGION 1..15: note = Description of Artificial Sequence: Cyclic peptide
HCLWQWTPQTHFVKL

SEQ ID NO: 270 - protein, 16 aa, synthetic construct
  REGION 1..16: note = Description of Artificial Sequence: Cyclic peptide
QCWWTLQVWSYPFHKH

SEQ ID NO: 271 - protein, 16 aa, synthetic construct
  REGION 1..16: note = Description of Artificial Sequence: Cyclic peptide
LCQLGVYTYVALFYKF

SEQ ID NO: 272 - protein, 16 aa, synthetic construct
  REGION 1..16: note = Description of Artificial Sequence: Cyclic peptide
QCDWVIWQWDPPYIKV

SEQ ID NO: 273 - protein, 16 aa, synthetic construct
  REGION 1..16: note = Description of Artificial Sequence: Cyclic peptide
PCWWATQIWTYPFYKV

SEQ ID NO: 274 - protein, 16 aa, synthetic construct
  REGION 1..16: note = Description of Artificial Sequence: Cyclic peptide
FCIYTFSRESGLLWKQ

SEQ ID NO: 275 - protein, 17 aa, synthetic construct
  REGION 1..17: note = Description of Artificial Sequence: Cyclic peptide
LCPLYAWQTLYQYGWKV

SEQ ID NO: 276 - protein, 17 aa, synthetic construct
  REGION 1..17: note = Description of Artificial Sequence: Cyclic peptide
ECIYTFDPQRHPVLVKV

SEQ ID NO: 277 - protein, 17 aa, synthetic construct
  REGION 1..17: note = Description of Artificial Sequence: Cyclic peptide
TCPVWAWHQAFQFGWKI

SEQ ID NO: 278 - protein, 18 aa, synthetic construct
  REGION 1..18: note = Description of Artificial Sequence: Cyclic peptide
ICPLYGDQGQAWQYGWKL

SEQ ID NO: 279 - protein, 18 aa, synthetic construct
  REGION 1..18: note = Description of Artificial Sequence: Cyclic peptide
QCLQKVGYLLWQFGWSKI

SEQ ID NO: 280 - protein, 18 aa, synthetic construct
  REGION 1..18: note = Description of Artificial Sequence: Cyclic peptide
PCPVWGDYGAVHQYGWKV

SEQ ID NO: 281 - protein, 18 aa, synthetic construct
  REGION 1..18: note = Description of Artificial Sequence: Cyclic peptide
YCVYTFDAQDVWRPLRKV

SEQ ID NO: 282 - protein, 19 aa, synthetic construct
  REGION 1..19: note = Description of Artificial Sequence: Cyclic peptide
FCIYSWNWNNLVRPEFRKV

SEQ ID NO: 283 - protein, 19 aa, synthetic construct
  REGION 1..19: note = Description of Artificial Sequence: Cyclic peptide
WCWLIPTPWPGVYQFSPKA

SEQ ID NO: 284 - protein, 19 aa, synthetic construct
  REGION 1..19: note = Description of Artificial Sequence: Cyclic peptide
QCRITLLTIYQWKYAWHKE

SEQ ID NO: 285 - protein, 19 aa, synthetic construct
  REGION 1..19: note = Description of Artificial Sequence: Cyclic peptide
QCSWWYVQVWTYPFHVLKG

SEQ ID NO: 286 - protein, 18 aa, synthetic construct
  REGION 1..18: note = Description of Artificial Sequence: Cyclic peptide
HCLWSLHSFYTFKAWAKI

SEQ ID NO: 287 - protein, 17 aa, synthetic construct
  REGION 1..17: note = Description of Artificial Sequence: Cyclic peptide
YCPFEVYSWWVPKWHKI

SEQ ID NO: 288 - protein, 19 aa, synthetic construct
  REGION 1..19: note = Description of Artificial Sequence: Cyclic peptide
LCHLVFQFNPDTGKLWPKY

SEQ ID NO: 289 - protein, 17 aa, synthetic construct
  REGION 1..17: note = Description of Artificial Sequence: Cyclic peptide
DCPWSVFSWYIPIYNKI

SEQ ID NO: 290 - protein, 20 aa, synthetic construct
  REGION 1..20: note = Description of Artificial Sequence: Cyclic peptide
FCVYTFDANAQSLDDALNKQ

SEQ ID NO: 291 - protein, 20 aa, synthetic construct
  REGION 1..20: note = Description of Artificial Sequence: Cyclic peptide
ICVYTFDAHAHSLDDALTKI

SEQ ID NO: 292 - protein, 20 aa, synthetic construct
  REGION 1..20: note = Description of Artificial Sequence: Cyclic peptide
ICVYTFDAHAHSLDAALNKI

SEQ ID NO: 293 - protein, 20 aa, synthetic construct
  REGION 1..20: note = Description of Artificial Sequence: Cyclic peptide
ICVYTFDAHAHSLDAALTKV

SEQ ID NO: 294 - protein, 20 aa, synthetic construct
  REGION 1..20: note = Description of Artificial Sequence: Cyclic peptide
ICVYTFDAHAHSLDAALTKQ

SEQ ID NO: 295 - protein, 20 aa, synthetic construct
  REGION 1..20: note = Description of Artificial Sequence: Cyclic peptide
ICVYTFDAHAHSLDAALNKV

SEQ ID NO: 296 - protein, 20 aa, synthetic construct
  REGION 1..20: note = Description of Artificial Sequence: Cyclic peptide
ICVYTFDAHAHSLDAALNKQ

SEQ ID NO: 297 - protein, 20 aa, synthetic construct
  REGION 1..20: note = Description of Artificial Sequence: Cyclic peptide
ICVYTFDAHAHSLHDALNKI

SEQ ID NO: 298 - protein, 20 aa, synthetic construct
  REGION 1..20: note = Description of Artificial Sequence: Cyclic peptide
ICVYTFDAHAHSLHDALTKV

SEQ ID NO: 299 - protein, 20 aa, synthetic construct
  REGION 1..20: note = Description of Artificial Sequence: Cyclic peptide
ICVYTFDAHAHSLHDALTKQ

SEQ ID NO: 300 - protein, 20 aa, synthetic construct
  REGION 1..20: note = Description of Artificial Sequence: Cyclic peptide
ICVYTFDAHAHSLHDALNKV

SEQ ID NO: 301 - protein, 20 aa, synthetic construct
  REGION 1..20: note = Description of Artificial Sequence: Cyclic peptide
ICVYTFDAHAHSLHDALNKQ

SEQ ID NO: 302 - protein, 20 aa, synthetic construct
  REGION 1..20: note = Description of Artificial Sequence: Cyclic peptide
ICVYTFDAHAHSLDDALNKI

SEQ ID NO: 303 - protein, 20 aa, synthetic construct
  REGION 1..20: note = Description of Artificial Sequence: Cyclic peptide
ICVYTFDAHAHSLDDALTKV

SEQ ID NO: 304 - protein, 20 aa, synthetic construct
  REGION 1..20: note = Description of Artificial Sequence: Cyclic peptide
ICVYTFDAHAHSLDDALTKQ

SEQ ID NO: 305 - protein, 20 aa, synthetic construct
  REGION 1..20: note = Description of Artificial Sequence: Cyclic peptide
ICVYTFDAHAHSLDDALNKV

SEQ ID NO: 306 - protein, 20 aa, synthetic construct
  REGION 1..20: note = Description of Artificial Sequence: Cyclic peptide
ICVYTFDAHAHSLDDALNKQ

SEQ ID NO: 307 - protein, 20 aa, synthetic construct
  REGION 1..20: note = Description of Artificial Sequence: Cyclic peptide
FCVYTFDAHAHSLDAALTKI

SEQ ID NO: 308 - protein, 20 aa, synthetic construct
  REGION 1..20: note = Description of Artificial Sequence: Cyclic peptide
FCVYTFDAHAHSLHDALTKI

SEQ ID NO: 309 - protein, 20 aa, synthetic construct
  REGION 1..20: note = Description of Artificial Sequence: Cyclic peptide
FCVYTFDAHAHSLDDALTKI

SEQ ID NO: 310 - protein, 20 aa, synthetic construct
  REGION 1..20: note = Description of Artificial Sequence: Cyclic peptide
ICVYTFDAHAQSLDAALTKI

SEQ ID NO: 311 - protein, 20 aa, synthetic construct
  REGION 1..20: note = Description of Artificial Sequence: Cyclic peptide
ICVYTFDAHAQSLHDALTKI

SEQ ID NO: 312 - protein, 20 aa, synthetic construct
  REGION 1..20: note = Description of Artificial Sequence: Cyclic peptide
ICVYTFDAHAQSLDDALTKI

SEQ ID NO: 313 - protein, 20 aa, synthetic construct
  REGION 1..20: note = Description of Artificial Sequence: Cyclic peptide
FCVYTFDAHAHSLDAALNKI

SEQ ID NO: 314 - protein, 20 aa, synthetic construct
  REGION 1..20: note = Description of Artificial Sequence: Cyclic peptide
FCVYTFDAHAHSLHDALNKI

SEQ ID NO: 315 - protein, 20 aa, synthetic construct
  REGION 1..20: note = Description of Artificial Sequence: Cyclic peptide
FCVYTFDAHAHSLDDALNKI

SEQ ID NO: 316 - protein, 20 aa, synthetic construct
  REGION 1..20: note = Description of Artificial Sequence: Cyclic peptide
FCVYTFDAHAHSLDAALTKQ

SEQ ID NO: 317 - protein, 20 aa, synthetic construct
  REGION 1..20: note = Description of Artificial Sequence: Cyclic peptide
FCVYTFDAHAHSLHDALTKQ

SEQ ID NO: 318 - protein, 20 aa, synthetic construct
  REGION 1..20: note = Description of Artificial Sequence: Cyclic peptide
FCVYTFDAHAHSLDDALTKQ

SEQ ID NO: 319 - protein, 20 aa, synthetic construct
  REGION 1..20: note = Description of Artificial Sequence: Cyclic peptide
FCVYTFDAHAHSLDAALNKQ

SEQ ID NO: 320 - protein, 20 aa, synthetic construct
  REGION 1..20: note = Description of Artificial Sequence: Cyclic peptide
FCVYTFDAHAHSLHDALNKQ

SEQ ID NO: 321 - protein, 20 aa, synthetic construct
  REGION 1..20: note = Description of Artificial Sequence: Cyclic peptide
FCVYTFDAHAHSLDDALNKQ

SEQ ID NO: 322 - protein, 19 aa, synthetic construct
  REGION 1..19: note = Description of Artificial Sequence: Cyclic peptide
CVYTFDAHAHSLDAALTKI

SEQ ID NO: 323 - protein, 20 aa, synthetic construct
  REGION 1..20: note = Description of Artificial Sequence: Cyclic peptide
ICVYTFDANAHSLDAALTKI

SEQ ID NO: 324 - protein, 20 aa, synthetic construct
  REGION 1..20: note = Description of Artificial Sequence: Cyclic peptide
ICVYTFDANAHSLHDALTKI

SEQ ID NO: 325 - protein, 20 aa, synthetic construct
  REGION 1..20: note = Description of Artificial Sequence: Cyclic peptide
ICVYTFDANAHSLDDALTKI

SEQ ID NO: 326 - protein, 20 aa, synthetic construct
  REGION 1..20: note = Description of Artificial Sequence: Cyclic peptide
IKVYTFDAHAHSLDAALTCI

SEQ ID NO: 327 - protein, 23 aa, synthetic construct
  REGION 1..23: note = Description of Artificial Sequence: Cyclic peptide
AXVWTFDRHAQEISQALHKVKKK

SEQ ID NO: 328 - protein, 23 aa, synthetic construct
  REGION 1..23: note = Description of Artificial Sequence: Cyclic peptide
AXVWTFDRHAQEISQALHXVKKK

SEQ ID NO: 329 - protein, 23 aa, synthetic construct
  REGION 1..23: note = Description of Artificial Sequence: Cyclic peptide
AXVWTFDRHAQEISQALHXVKKK

SEQ ID NO: 330 - protein, 23 aa, synthetic construct
  REGION 1..23: note = Description of Artificial Sequence: Cyclic peptide
AXVWTFDRHAQEISQALHXVKKK

SEQ ID NO: 331 - protein, 23 aa, synthetic construct
  REGION 1..23: note = Description of Artificial Sequence: Cyclic peptide
AKVWTFDRHAQEISQALHXVKKK

SEQ ID NO: 332 - protein, 23 aa, synthetic construct
  REGION 1..23: note = Description of Artificial Sequence: Cyclic peptide
AXVWTFDRHAQEISQALHXVKKK

SEQ ID NO: 333 - protein, 23 aa, synthetic construct
  REGION 1..23: note = Description of Artificial Sequence: Cyclic peptide
AXVWTFDRHAQEISQALHXVKKK

SEQ ID NO: 334 - protein, 23 aa, synthetic construct
  REGION 1..23: note = Description of Artificial Sequence: Cyclic peptide
AXVWTFDRHAQEISQALHXVKKK

SEQ ID NO: 335 - protein, 23 aa, synthetic construct
  REGION 1..23: note = Description of Artificial Sequence: Cyclic peptide
ACVWTFDRHAQEISQALHKVKKK

SEQ ID NO: 336 - protein, 23 aa, synthetic construct
  REGION 1..23: note = Description of Artificial Sequence: Cyclic peptide
ACVWTFDRHAQEISQALHCVKKK

SEQ ID NO: 337 - protein, 23 aa, synthetic construct
  REGION 1..23: note = Description of Artificial Sequence: Cyclic peptide
FXVYTFDAHAHSLDAALNXIKKK

SEQ ID NO: 338 - protein, 23 aa, synthetic construct
  REGION 1..23: note = Description of Artificial Sequence: Cyclic peptide
FXVYTFDAHAHSLDAALNXIKKK

SEQ ID NO: 339 - protein, 23 aa, synthetic construct
  REGION 1..23: note = Description of Artificial Sequence: Cyclic peptide
FXVYTFDAHAHSLDAALNXIKKK

SEQ ID NO: 340 - protein, 23 aa, synthetic construct
  REGION 1..23: note = Description of Artificial Sequence: Cyclic peptide
FXVYTFDAHAHSXDAALNXIKKK

SEQ ID NO: 341 - protein, 22 aa, synthetic construct
  REGION 1..22: note = Description of Artificial Sequence: Cyclic peptide
XVYTFDAHAHSLDAALNXIKKK

SEQ ID NO: 342 - protein, 22 aa, synthetic construct
  REGION 1..22: note = Description of Artificial Sequence: Cyclic peptide
FXVYTFDAHAHSLDAALNXKKK

SEQ ID NO: 343 - protein, 55 aa, synthetic construct
  REGION 1..55: note = Description of Artificial Sequence: Cyclic peptide
ACVWTFDRHAQEISQALHKVGSGSGSSGSGSSGSSACVWTFDRHAQEISQALHKV

SEQ ID NO: 344 - protein, 40 aa, synthetic construct
  REGION 1..40: note = Description of Artificial Sequence: Cyclic peptide
ACVWTFDRHAQEISQALHKVACVWTFDRHAQEISQALHKV

SEQ ID NO: 345 - protein, 40 aa, synthetic construct
  REGION 1..40: note = Description of Artificial Sequence: Cyclic peptide
FXVYTFDAHAHSLDAALNXIFXVYTFDAHAHSLDAALNXI

SEQ ID NO: 346 - protein, 40 aa, synthetic construct; identical to SEQ ID NO: 345
  REGION 1..40: note = Description of Artificial Sequence: Cyclic peptide